European Patent Application EP 4 162 952 A1, published April 12, 2023. Title: Agent for preventing or treating RNA virus-related disease. Applicant: Kyoto University Nagasaki University. The sequence listing filed with the application follows.

SEQUENCE LISTING (4 sequences)

SEQ ID NO: 1 - DNA, 20 bp, Artificial Sequence
  Synthesized oligonucleotide
ggacgacggcaactacaaga

SEQ ID NO: 2 - DNA, 20 bp, Artificial Sequence
  Synthesized oligonucleotide
ttgtactccagcttgtgccc

SEQ ID NO: 3 - DNA, 18 bp, Artificial Sequence
  Synthesized oligonucleotide
tccactggcgtcttcacc

SEQ ID NO: 4 - DNA, 21 bp, Artificial Sequence
  Synthesized oligonucleotide
ggcagagatgatgaccctttt